European Patent Application EP 4 667 569 A1, published December 24, 2025. Title: Multivalent binding nucleic acid agent. Applicant: National University Corporation Tokyo Medical and Dental University. Application JP. The sequence listing filed with the application follows.

SEQUENCE LISTING (18 sequences)

SEQ ID NO: 1 - RNA, 12 nt, synthetic construct
  source 1..12: mol_type = other RNA
  misc_feature 1..12: note = 2'-O-methyl RNA
tgtgtgtgtgtg

SEQ ID NO: 2 - RNA, 24 nt, synthetic construct
  source 1..24: mol_type = other RNA
  misc_feature 1..24: note = 2'-O-methyl RNA
tgtgtgtgtgtgtgtgtgtgtgtg

SEQ ID NO: 3 - RNA, 36 nt, synthetic construct
  source 1..36: mol_type = other RNA
  misc_feature 1..36: note = 2'-O-methyl RNA
tgtgtgtgtgtgaaaaaaaaaaaatgtgtgtgtgtg

SEQ ID NO: 4 - RNA, 36 nt, synthetic construct; identical to SEQ ID NO: 3
  source 1..36: mol_type = other RNA
  misc_feature order(1..12,25..36): note = 2'-O-methyl RNA
  misc_feature 13..24: note = LNA

SEQ ID NO: 5 - DNA, 12 bp, synthetic construct
  source 1..12: mol_type = other DNA
tttttttttttt

SEQ ID NO: 6 - RNA, 12 nt, synthetic construct
  source 1..12: mol_type = other RNA
gtgtgaatgaat

SEQ ID NO: 7 - RNA, 34 nt, synthetic construct
  source 1..34: mol_type = other RNA
gagagagcgcgtgcagagacttggtggtgcataa

SEQ ID NO: 8 - RNA, 24 nt, synthetic construct
  source 1..24: mol_type = other RNA
tgtgtgtgtgtgtttttttttttt

SEQ ID NO: 9 - RNA, 24 nt, synthetic construct
  source 1..24: mol_type = other RNA
tgtgtgtgtgtgaaaaaaaaaaaa

SEQ ID NO: 10 - RNA, 48 nt, synthetic construct
  source 1..48: mol_type = other RNA
  misc_feature 1..48: note = 2'-O-methyl RNA
tgtgtgtgtgtgaaaaaaaaaaaaaaaaaaaaaaaatgtgtgtgtgtg

SEQ ID NO: 11 - RNA, 72 nt, synthetic construct
  source 1..72: mol_type = other RNA
  misc_feature 1..72: note = 2'-O-methyl RNA
tgtgtgtgtgtgaaaaaaaaaaaaaaaaaaaaaaaaaaaaaaaaaaaaaaaaaaaaaaaatgtgtgtgtgtg

SEQ ID NO: 12 - RNA, 60 nt, synthetic construct
  source 1..60: mol_type = other RNA
  misc_feature 1..60: note = 2'-O-methyl RNA
tgtgtgtgtgtgaaaaaaaaaaaatgtgtgtgtgtgaaaaaaaaaaaatgtgtgtgtgtg

SEQ ID NO: 13 - DNA, 24 bp, synthetic construct
  source 1..24: mol_type = other DNA
tttttttttttttttttttttttt

SEQ ID NO: 14 - DNA, 48 bp, synthetic construct
  source 1..48: mol_type = other DNA
tttttttttttttttttttttttttttttttttttttttttttttttt

SEQ ID NO: 15 - DNA, 22 bp, synthetic construct
  misc_feature 13..22: note = DNA
  misc_feature 1..12: note = 2'-O-methyl RNA
  source 1..22: mol_type = other DNA
tgtgtgtgtgtgctgcgcgagc

SEQ ID NO: 16 - DNA, 22 bp, synthetic construct
  misc_feature 13..22: note = DNA
  misc_feature 1..12: note = 2'-O-methyl RNA
  source 1..22: mol_type = other DNA
tgtgtgtgtgtggctcgcgcag

SEQ ID NO: 17 - DNA, 22 bp, synthetic construct
  misc_feature 13..22: note = DNA
  misc_feature 1..12: note = 2'-O-methyl RNA
  source 1..22: mol_type = other DNA
gacgcgctcgtgtgtgtgtgtg

SEQ ID NO: 18 - DNA, 22 bp, synthetic construct
  misc_feature 13..22: note = DNA
  misc_feature 1..12: note = 2'-O-methyl RNA
  source 1..22: mol_type = other DNA
cgagcgcgtctgtgtgtgtgtg